European Patent Specification EP 3 436 601 B1, published March 29, 2023. Title: Cytidine Deaminase expression level in cancer as a new therapeutic target. Applicant: Institut Curie. The sequence listing filed with the application follows.

SEQUENCE LISTING (16 sequences)

SEQ ID NO: 1 - DNA, 21 bp, Artificial Sequence
  Primer F1 of the promoter and exon 1
aacgggatgacttattgaggt

SEQ ID NO: 2 - DNA, 20 bp, Artificial Sequence
  Primer R1 of the promoter and exon 1
catcttcctctgacccacca

SEQ ID NO: 3 - DNA, 19 bp, Artificial Sequence
  Primer F2 of the exon 2
attgccctgtccttctccc

SEQ ID NO: 4 - DNA, 20 bp, Artificial Sequence
  Primer R2 of the exon 2
tatcctcagcactcatccca

SEQ ID NO: 5 - DNA, 20 bp, Artificial Sequence
  Primer F3 of the exon 3
ccaaatcaggaacagaccga

SEQ ID NO: 6 - DNA, 20 bp, Artificial Sequence
  Primer R3 of the exon 3
cacaaagcagacactcactc

SEQ ID NO: 7 - DNA, 21 bp, Artificial Sequence
  Primer F4 of the exon 4
agcattctttcgtttcctcct

SEQ ID NO: 8 - DNA, 19 bp, Artificial Sequence
  Primer R4 of the exon 4
atctccacaccctcctcac

SEQ ID NO: 9 - DNA, 19 bp, Artificial Sequence
  Primer F of CDA
ccctacagtcactttcctg

SEQ ID NO: 10 - DNA, 20 bp, Artificial Sequence
  Primer R of CDA
cgggtagcaggcattttcta

SEQ ID NO: 11 - DNA, 24 bp, Artificial Sequence
  Primer F of GAPDH
gaaatcccatcaccatcttccagg

SEQ ID NO: 12 - DNA, 20 bp, Artificial Sequence
  Primer R of GAPDH
gagccccagccttctccatg

SEQ ID NO: 13 - DNA, 21 bp, Artificial Sequence
  Primer F of TBP
tgcacaggagccaagagtgaa

SEQ ID NO: 14 - DNA, 20 bp, Artificial Sequence
  Primer R of TBP
cacatcacagctccccacca

SEQ ID NO: 15 - DNA, 19 bp, Artificial Sequence
  Primer ESR1 Forward
ccggctccgcaaatgctac

SEQ ID NO: 16 - DNA, 21 bp, Artificial Sequence
  Primer ESR1 Reverse
aaggttggcagctctcatgtc